European Patent Specification EP 3 913 058 B1, published January 1, 2025. Title: OLIGONUCLEOTIDES COMPRISING MODIFIED NUCLEOSIDES. Applicant: SOMALOGIC, INC. Application Unknown, filed herewith. The sequence listing filed with the application follows.

SEQUENCE LISTING (83 sequences)

SEQ ID NO: 1 - DNA, 79 bp, Artificial Sequence
  source: /note="Description of Artificial Sequence: Synthetic oligonucleotide"
  modified_base (34)..(63): a, c, t, g, unknown or other
aattttttttctctttctcttctctctttctccnnnnnnnnnnnnnnnnnnnnnnnnnnnnnngacccacccagcgtgg

SEQ ID NO: 2 - DNA, 24 bp, Artificial Sequence
  source: /note="Description of Artificial Sequence: Synthetic oligonucleotide"
atatatatccacgctgggtgggtc

SEQ ID NO: 3 - DNA, 33 bp, Artificial Sequence
  source: /note="Description of Artificial Sequence: Synthetic oligonucleotide"
aattttttttctctttctcttctctctttctcc

SEQ ID NO: 4 - DNA, 30 bp, Artificial Sequence
  source: /note="Description of Artificial Sequence: Synthetic oligonucleotide"
aagttccggccgcctcggggtccctgccaa

SEQ ID NO: 5 - DNA, 30 bp, Artificial Sequence
  source: /note="Description of Artificial Sequence: Synthetic oligonucleotide"
atacctgggattccggccatttgcgcagtt

SEQ ID NO: 6 - DNA, 30 bp, Artificial Sequence
  source: /note="Description of Artificial Sequence: Synthetic oligonucleotide"
tgaagttccggccgtgcgcatggtacccat

SEQ ID NO: 7 - DNA, 30 bp, Artificial Sequence
  source: /note="Description of Artificial Sequence: Synthetic oligonucleotide"
tttgtgcttccggcctagcgcagatatcct

SEQ ID NO: 8 - DNA, 29 bp, Artificial Sequence
  source: /note="Description of Artificial Sequence: Synthetic oligonucleotide"
ataggttccggccttgcgctgtttagaca

SEQ ID NO: 9 - DNA, 30 bp, Artificial Sequence
  source: /note="Description of Artificial Sequence: Synthetic oligonucleotide"
tagatgcctggtatttccggccttgcgcat

SEQ ID NO: 10 - DNA, 30 bp, Artificial Sequence
  source: /note="Description of Artificial Sequence: Synthetic oligonucleotide"
tagtgccctgatctattccggccaagccca

SEQ ID NO: 11 - DNA, 31 bp, Artificial Sequence
  source: /note="Description of Artificial Sequence: Synthetic oligonucleotide"
tttgcccctggttacgttccggcctggcgca

SEQ ID NO: 12 - DNA, 30 bp, Artificial Sequence
  source: /note="Description of Artificial Sequence: Synthetic oligonucleotide"
atgccgttccggcctagcgctcgttaccca

SEQ ID NO: 13 - DNA, 30 bp, Artificial Sequence
  source: /note="Description of Artificial Sequence: Synthetic oligonucleotide"
tgaccacctgtccaattccggcctagcgca

SEQ ID NO: 14 - DNA, 30 bp, Artificial Sequence
  source: /note="Description of Artificial Sequence: Synthetic oligonucleotide"
taccaggtattccggccgagcgctgctata

SEQ ID NO: 15 - DNA, 30 bp, Artificial Sequence
  source: /note="Description of Artificial Sequence: Synthetic oligonucleotide"
gagcccagttacttccggccttgcattgta

SEQ ID NO: 16 - DNA, 29 bp, Artificial Sequence
  source: /note="Description of Artificial Sequence: Synthetic oligonucleotide"
aagagtttccggcctaccgcattcaccct

SEQ ID NO: 17 - DNA, 34 bp, Artificial Sequence
  source: /note="Description of Artificial Sequence: Synthetic oligonucleotide"
acagtcccacagtttaattccggccgtagccgct

SEQ ID NO: 18 - DNA, 30 bp, Artificial Sequence
  source: /note="Description of Artificial Sequence: Synthetic oligonucleotide"
ataccagggtcgttccggccaagcgctgtt

SEQ ID NO: 19 - DNA, 30 bp, Artificial Sequence
  source: /note="Description of Artificial Sequence: Synthetic oligonucleotide"
gagttccggcctagcgcagaagccctggat

SEQ ID NO: 20 - DNA, 30 bp, Artificial Sequence
  source: /note="Description of Artificial Sequence: Synthetic oligonucleotide"
ttttccaggaattccggccaagcgctgtga

SEQ ID NO: 21 - DNA, 30 bp, Artificial Sequence
  source: /note="Description of Artificial Sequence: Synthetic oligonucleotide"
aattacctgaggattccggccaagcgcaga

SEQ ID NO: 22 - DNA, 30 bp, Artificial Sequence
  source: /note="Description of Artificial Sequence: Synthetic oligonucleotide"
ctgcgttacgccttccggcctggctgatag

SEQ ID NO: 23 - DNA, 30 bp, Artificial Sequence
  source: /note="Description of Artificial Sequence: Synthetic oligonucleotide"
tacctgagttatgtattccggccgtgcgca

SEQ ID NO: 24 - DNA, 30 bp, Artificial Sequence
  source: /note="Description of Artificial Sequence: Synthetic oligonucleotide"
caaagcattccggccttgcgcagtagccct

SEQ ID NO: 25 - DNA, 30 bp, Artificial Sequence
  source: /note="Description of Artificial Sequence: Synthetic oligonucleotide"
gtagttccagattgattccggccttgcgct

SEQ ID NO: 26 - DNA, 30 bp, Artificial Sequence
  source: /note="Description of Artificial Sequence: Synthetic oligonucleotide"
aatactccaggtgagttccggccaagcgct

SEQ ID NO: 27 - RNA, 30 nt, Artificial Sequence
  source: /note="Description of Artificial Sequence: Synthetic oligonucleotide"
guuaucgcaaugugcgcccgggugcccgcc

SEQ ID NO: 28 - RNA, 30 nt, Artificial Sequence
  source: /note="Description of Artificial Sequence: Synthetic oligonucleotide"
ugugcccggauauuaacuguuccgagcagu

SEQ ID NO: 29 - RNA, 30 nt, Artificial Sequence
  source: /note="Description of Artificial Sequence: Synthetic oligonucleotide"
uguuuaugcacaugcccgcgaugacaguaa

SEQ ID NO: 30 - RNA, 30 nt, Artificial Sequence
  source: /note="Description of Artificial Sequence: Synthetic oligonucleotide"
agugugauuaugcacuugcccgcauuuggu

SEQ ID NO: 31 - RNA, 30 nt, Artificial Sequence
  source: /note="Description of Artificial Sequence: Synthetic oligonucleotide"
uauagaacauaaugcacaugcccgcauacu

SEQ ID NO: 32 - RNA, 30 nt, Artificial Sequence
  source: /note="Description of Artificial Sequence: Synthetic oligonucleotide"
uaucaguuuaugcacgugcccgcgaugacu

SEQ ID NO: 33 - RNA, 30 nt, Artificial Sequence
  source: /note="Description of Artificial Sequence: Synthetic oligonucleotide"
gacuacgagggaugaugcacaugcccgcau

SEQ ID NO: 34 - RNA, 30 nt, Artificial Sequence
  source: /note="Description of Artificial Sequence: Synthetic oligonucleotide"
auaaugauuaugcacaugcccgcaugucau

SEQ ID NO: 35 - RNA, 30 nt, Artificial Sequence
  source: /note="Description of Artificial Sequence: Synthetic oligonucleotide"
ggcaucgugugcccgauuuucuaaccggga

SEQ ID NO: 36 - RNA, 30 nt, Artificial Sequence
  source: /note="Description of Artificial Sequence: Synthetic oligonucleotide"
gccgaauuuaugcaccugcccgcaugauuc

SEQ ID NO: 37 - RNA, 29 nt, Artificial Sequence
  source: /note="Description of Artificial Sequence: Synthetic oligonucleotide"
ccaaucaugacacaugcccggaugauacu

SEQ ID NO: 38 - RNA, 30 nt, Artificial Sequence
  source: /note="Description of Artificial Sequence: Synthetic oligonucleotide"
uacgaugcccggauauugacuguuccgucg

SEQ ID NO: 39 - RNA, 31 nt, Artificial Sequence
  source: /note="Description of Artificial Sequence: Synthetic oligonucleotide"
cguagcgacgggcguggcaugcccggccccc

SEQ ID NO: 40 - RNA, 30 nt, Artificial Sequence
  source: /note="Description of Artificial Sequence: Synthetic oligonucleotide"
uggugagagugcccggauauuaacuguucc

SEQ ID NO: 41 - RNA, 30 nt, Artificial Sequence
  source: /note="Description of Artificial Sequence: Synthetic oligonucleotide"
ucaaaggccgugugcccgauuuucuaaccg

SEQ ID NO: 42 - RNA, 30 nt, Artificial Sequence
  source: /note="Description of Artificial Sequence: Synthetic oligonucleotide"
uuucgaaguugagcguggcaauacuugccc

SEQ ID NO: 43 - RNA, 30 nt, Artificial Sequence
  source: /note="Description of Artificial Sequence: Synthetic oligonucleotide"
cguguuuaugcacuugcccgcgauuacacc

SEQ ID NO: 44 - RNA, 30 nt, Artificial Sequence
  source: /note="Description of Artificial Sequence: Synthetic oligonucleotide"
aacguacuuuaaggccuauugaggaaacuc

SEQ ID NO: 45 - RNA, 30 nt, Artificial Sequence
  source: /note="Description of Artificial Sequence: Synthetic oligonucleotide"
cacuuuaagaccuauugcggagacccuggg

SEQ ID NO: 46 - RNA, 30 nt, Artificial Sequence
  source: /note="Description of Artificial Sequence: Synthetic oligonucleotide"
cgugcuuuaagaccuguugagaugcgcuca

SEQ ID NO: 47 - RNA, 30 nt, Artificial Sequence
  source: /note="Description of Artificial Sequence: Synthetic oligonucleotide"
acuuuaagaccuguugagggccucgggaau

SEQ ID NO: 48 - RNA, 30 nt, Artificial Sequence
  source: /note="Description of Artificial Sequence: Synthetic oligonucleotide"
gccgguguuuaagaacuguuggggcacuuc

SEQ ID NO: 49 - RNA, 30 nt, Artificial Sequence
  source: /note="Description of Artificial Sequence: Synthetic oligonucleotide"
gcgcacuuuaagaccuauuggggagaacuc

SEQ ID NO: 50 - RNA, 30 nt, Artificial Sequence
  source: /note="Description of Artificial Sequence: Synthetic oligonucleotide"
uuuaaggccuguugaggaccucggcaugaa

SEQ ID NO: 51 - RNA, 30 nt, Artificial Sequence
  source: /note="Description of Artificial Sequence: Synthetic oligonucleotide"
caacuuuaaggccuguugggagagcccuug

SEQ ID NO: 52 - RNA, 30 nt, Artificial Sequence
  source: /note="Description of Artificial Sequence: Synthetic oligonucleotide"
gaauaccacgcuuuaagaccuauuggaucg

SEQ ID NO: 53 - RNA, 30 nt, Artificial Sequence
  source: /note="Description of Artificial Sequence: Synthetic oligonucleotide"
gagaacuuuaagaccuauugagggccucug

SEQ ID NO: 54 - RNA, 29 nt, Artificial Sequence
  source: /note="Description of Artificial Sequence: Synthetic oligonucleotide"
cgacuuuaaggccuauugggggacucgac

SEQ ID NO: 55 - RNA, 30 nt, Artificial Sequence
  source: /note="Description of Artificial Sequence: Synthetic oligonucleotide"
gaacacuuuaagaccuguugggaagcgucu

SEQ ID NO: 56 - RNA, 30 nt, Artificial Sequence
  source: /note="Description of Artificial Sequence: Synthetic oligonucleotide"
acuuuaaggccuguugaggaaaccgucuga

SEQ ID NO: 57 - RNA, 30 nt, Artificial Sequence
  source: /note="Description of Artificial Sequence: Synthetic oligonucleotide"
agcuuuaagaccuguugagaauucgacaaa

SEQ ID NO: 58 - RNA, 30 nt, Artificial Sequence
  source: /note="Description of Artificial Sequence: Synthetic oligonucleotide"
agcuuuaagaccuguugagcagccucgacc

SEQ ID NO: 59 - RNA, 30 nt, Artificial Sequence
  source: /note="Description of Artificial Sequence: Synthetic oligonucleotide"
gaaggucaaguggcacuuuaaggccuguuc

SEQ ID NO: 60 - RNA, 30 nt, Artificial Sequence
  source: /note="Description of Artificial Sequence: Synthetic oligonucleotide"
aaaccacuuuaagaccuguuggggcacucu

SEQ ID NO: 61 - RNA, 30 nt, Artificial Sequence
  source: /note="Description of Artificial Sequence: Synthetic oligonucleotide"
aaaccuuuaagaccuauugaggugggcuca

SEQ ID NO: 62 - RNA, 30 nt, Artificial Sequence
  source: /note="Description of Artificial Sequence: Synthetic oligonucleotide"
uaggcgcuuuaagaccuauugagggacucc

SEQ ID NO: 63 - RNA, 30 nt, Artificial Sequence
  source: /note="Description of Artificial Sequence: Synthetic oligonucleotide"
gugacgcuuuaagaccuauuagggcacuuc

SEQ ID NO: 64 - RNA, 30 nt, Artificial Sequence
  source: /note="Description of Artificial Sequence: Synthetic oligonucleotide"
gaaaccacuuuaagaccuauugagagacuc

SEQ ID NO: 65 - RNA, 30 nt, Artificial Sequence
  source: /note="Description of Artificial Sequence: Synthetic oligonucleotide"
gaaacuuuaagaccuauugagcaggaacuc

SEQ ID NO: 66 - skipped

SEQ ID NO: 67 - RNA, 30 nt, Artificial Sequence
  source: /note="Description of Artificial Sequence: Synthetic oligonucleotide"
cgacuuuaagaccuguugaaagucgcgggg

SEQ ID NO: 68 - RNA, 32 nt, Artificial Sequence
  source: /note="Description of Artificial Sequence: Synthetic oligonucleotide"
acuuuaagaccuguugagaccggcucggacau

SEQ ID NO: 69 - RNA, 30 nt, Artificial Sequence
  source: /note="Description of Artificial Sequence: Synthetic oligonucleotide"
gaacuuuaagaccuguugaggaccaucacg

SEQ ID NO: 70 - RNA, 30 nt, Artificial Sequence
  source: /note="Description of Artificial Sequence: Synthetic oligonucleotide"
acguggagucggacacuuuaaggccuguuc

SEQ ID NO: 71 - RNA, 30 nt, Artificial Sequence
  source: /note="Description of Artificial Sequence: Synthetic oligonucleotide"
ucgcgacuuuaaggccuauugugggacucu

SEQ ID NO: 72 - RNA, 30 nt, Artificial Sequence
  source: /note="Description of Artificial Sequence: Synthetic oligonucleotide"
gcuuuaaggccuauugagaucggcucgggu

SEQ ID NO: 73 - RNA, 30 nt, Artificial Sequence
  source: /note="Description of Artificial Sequence: Synthetic oligonucleotide"
gacuuuaaggccuguugaaggucgagaguu

SEQ ID NO: 74 - RNA, 29 nt, Artificial Sequence
  source: /note="Description of Artificial Sequence: Synthetic oligonucleotide"
aacgaucuuuaaggccuguuaggggcuuc

SEQ ID NO: 75 - RNA, 30 nt, Artificial Sequence
  source: /note="Description of Artificial Sequence: Synthetic oligonucleotide"
caagcugccucgcacuuuaagacguguugg

SEQ ID NO: 76 - RNA, 30 nt, Artificial Sequence
  source: /note="Description of Artificial Sequence: Synthetic oligonucleotide"
accguguuuaagaacuguuggggggaacuc

SEQ ID NO: 77 - RNA, 36 nt, Artificial Sequence
  source: /note="Description of Artificial Sequence: Synthetic oligonucleotide"
gaauaccacgcuuuaagaccuauugagaugcgcuca

SEQ ID NO: 78 - RNA, 30 nt, Artificial Sequence
  source: /note="Description of Artificial Sequence: Synthetic oligonucleotide"
uaagccugagaaaccacuuuaagaccuuuu

SEQ ID NO: 79 - RNA, 30 nt, Artificial Sequence
  source: /note="Description of Artificial Sequence: Synthetic oligonucleotide"
cgaacuuuaagaccuguugagcagcucuuc

SEQ ID NO: 80 - RNA, 30 nt, Artificial Sequence
  source: /note="Description of Artificial Sequence: Synthetic oligonucleotide"
agaaucuuuaaggccugucgagaccucgag

SEQ ID NO: 81 - DNA, 15 bp, Artificial Sequence
  source: /note="Description of Artificial Sequence: Synthetic oligonucleotide"
  misc_feature (1)..(1): /note="May or may not be present"
  misc_feature (15)..(15): /note="May or may not be present"
  source: /note="See specification as filed for detailed description of substitutions and preferred embodiments"
scccaagrmccrccv

SEQ ID NO: 82 - DNA, 10 bp, Artificial Sequence
  source: /note="Description of Artificial Sequence: Synthetic oligonucleotide"
aatttttttt

SEQ ID NO: 83 - RNA, 15 nt, Artificial Sequence
  source: /note="Description of Artificial Sequence: Synthetic oligonucleotide"
cuuuaaggccuauug